European Patent Specification EP 4 121 003 B1, published August 6, 2025. Title: LIQUID FORMULATIONS OF GLUCAGON ANALOGUES. Applicant: ZEALAND PHARMA A/S. Application 20163408.6. The sequence listing filed with the application follows.

SEQUENCE LISTING (1 sequence)

SEQ ID NO: 1 - protein, 29 aa, Artificial Sequence
  Artificial sequence
  MISC_FEATURE (16)..(16): Xaa = Aib
HSQGTFTSDYSKYLDXARAEEFVKWLEST